European Patent Specification EP 3 578 667 B1, published October 4, 2023. Title: Methods For Characterizing DNA Sequence Composition in a Genome. Applicant: Pioneer Hi-Bred International, Inc. The sequence listing filed with the application follows.

SEQUENCE LISTING (8 sequences)

SEQ ID NO: 1 - DNA, 50 bp, Artificial Sequence
  Putative Junction Sequence
aagttgtaatttaaattgaatacagaagggctccggccccggcgccacca

SEQ ID NO: 2 - DNA, 50 bp, Artificial Sequence
  Putative Junction Sequence
aagttgtaatttaaattgaatagagaagggctccggccccggcgccacca

SEQ ID NO: 3 - DNA, 50 bp, Artificial Sequence
  Putative Junction Sequence
aagttgtaatttaaattgaatacagaaggactccggccccggcgccacca

SEQ ID NO: 4 - DNA, 50 bp, Artificial Sequence
  Putative Junction Sequence
aagttgtaatttaaattgaatacagaggggctccggccccggcgccacca

SEQ ID NO: 5 - DNA, 50 bp, Artificial Sequence
  Putative Junction Sequence
aagttgtaatttaaattgaatacagaagggctccggccccggcaccacca

SEQ ID NO: 6 - DNA, 50 bp, Artificial Sequence
  Putative Junction Sequence
aagttgtaatttaagttgaatacagaagggctccggccccggcgccacca

SEQ ID NO: 7 - DNA, 50 bp, Artificial Sequence
  Putative Junction Sequence
aagttgtaatttaaattgaatacagaagggctccggtcccggcgccacca

SEQ ID NO: 8 - DNA, 50 bp, Artificial Sequence
  Putative Junction Sequence
agttgtaatttaaattgaatacagaagggctccggccccggcgccaccaa